European Patent Specification EP 4 050 034 B1, published May 8, 2024. Title: CD3 Binding Antibodies. Applicant: Teneobio, Inc. The sequence listing filed with the application follows.

SEQUENCE LISTING (22 sequences)

SEQ ID NO: 1 - protein, 123 aa, Homo sapiens
EVQLVESGGGLVQPGRSLRLSCAASGFTFDDYAMHWVRQAPGKGLEWVSGISWNSGSIGYADSVKGRFTISRDNAKNSLYLQMNSLRAEDTALYYCAKDSRGYGDYRLGGAYWGQGTLVTVSS

SEQ ID NO: 2 - protein, 123 aa, Homo sapiens
EVQLVESGGGLVKPGGSLRLSCAASGFTFDDYAMHWVRQAPGKGLEWVSGISWNSGSIGYADSVKGRFTISRDNAKNSLYLQMNSLRAEDTALYYCAKDSRGYGDYRLGGAYWGQGTLVTVSS

SEQ ID NO: 3 - protein, 123 aa, Homo sapiens
EVQLVESGGGLVQPGRSLRLSCAASGFTFDDYAMHWVRQAPGKGLEWVSGISWNSGSIGYADSVKGRFTISRDNAKKSLYLQMNSLRAEDTALYYCAKDSRGYGDYSRGGAYWGQGTLVTVSS

SEQ ID NO: 4 - protein, 123 aa, Homo sapiens
EVQLVESGGGLVQPGRSLRLSCAASGFTFDDYAMHWVRQAPGKGLEWVSGISWNSGSIGYADSVKGRFTISRDNAKNSLYLQMNSLRPEDTALYYCAKDSRGYGDYSLGGAYWGQGTLVTVSS

SEQ ID NO: 5 - protein, 123 aa, Homo sapiens
EVQLVESGGGLVQPGRSLRLSCAASGFTFDDYAMHWVRQAPGKGLEWVSGISWNSGSIGYADSVKGRFTISRDNAKNSLYLQMNSLRAEDTALYYCAKDSRGYGDYSLGGAYWGQGTLVTVSS

SEQ ID NO: 6 - protein, 123 aa, Homo sapiens
EVQLVESGGGLVQPGRSLRLSCAASGFTFANYAMHWVRQAPGKGLEWVSGISWNSGSIDYADSVKGRFTISRDNAKNSLYLQMNSLRAEDTALYYCAKDSRGYGDYSRGGAYWGQGTLVTVSS

SEQ ID NO: 7 - protein, 123 aa, Homo sapiens
EVQLVESGGGLVQPGRSLRLSCAASGFTFNNYAMHWVRQAPGKGLEWVSGISWNSGSIGYADSVKGRFTISRDNAKNSLYLQMNSLRGEDTALYYCAKDSRGYGDYSRGGAYWGQGTLVTVSS

SEQ ID NO: 8 - protein, 123 aa, Homo sapiens
EVQLVESGGGLVQPGGSLRLSCAASGFTFADYAMHWVRQAPGKGLEWVSGISWNSGSIGYADSVKGRFTISRDNAKNSLYLQMNSLRAEDTALYYCAKDSRGYGDYSRGGAYWGQGTLVTVSS

SEQ ID NO: 9 - protein, 123 aa, Homo sapiens
EVQLVESGGGLVQPGRSLRLSCAASGFTFDNYAMHWVRQAPGKGLEWVSGISWNSGSIGYADSVKGRFTISRDNAKKSLYLQMNSLRAEDTALYYCAKDSRGYGDYSRGGAYWGQGTLVTVSS

SEQ ID NO: 10 - protein, 123 aa, Homo sapiens
EVQLVESGGGLVQPGRSLRLSCAASGFTFDNYAMHWVRQAPGKGLEWVSGISWNSGSIGYADSVKGRFTISRDNAKNSLYLQMNSLRAEDTALYYCAKDSRGYGDYSRGGAYWGQGTLVTVSS

SEQ ID NO: 11 - protein, 123 aa, Homo sapiens
EVQLVESGGGLVQPGRSLRLSCAASGFTFDDYAMHWVRQAPGKGLEWVSGISWNSGSIGYADSVKGRFTISRDNAKNSLYLQMNSLRAEDTALYYCAKDSRGYGDYSRGGAYWGQGTLVTVSS

SEQ ID NO: 12 - protein, 123 aa, Homo sapiens
EVQLVESGGGLVQPGRSLRLSCAASGFTFDDYAMHWVRQAPGKGLEWVSGISWNSGSIGYADSVKGRFTISRDNAKNSLYLQMNSLRPEDTALYYCAKDSRGYGSYSRGGAYWGQGTLVTVSS

SEQ ID NO: 13 - protein, 123 aa, Homo sapiens
EVQLVESGGGLVQPGRSLRLSCAASGFTFHNYAMHWVRQAPGKGLEWVSGISWNSGSIGYADSVKGRFTISRDNAKNSLYLQMNSLRAEDTALYYCAKDSRGYGDYSLGGAYWGQGTLVTVSS

SEQ ID NO: 14 - protein, 123 aa, Homo sapiens
EVQLVESGGGLVQPGGSLRLSCAASGFTFDDYAMHWVRQAPGKGLEWVSGISWNSGSIGYADSVKGRFTISRDNAKNSLYLQMNSLRAEDTALYYCAKDSRGYGDYSRGGAYCGQGTLVTVSS

SEQ ID NO: 15 - protein, 123 aa, Homo sapiens
EVQLVESGGGLVQPGRSLRLSCAASGFTFDNYAMHWVRQAPGKGLEWVSGISWNSGSIGYADSVKGRFTISRDNAKKSLYLQMNSLRAEDTALYYCAKDSRGYGDYSLGGAYWGQGTLVTVSS

SEQ ID NO: 16 - protein, 123 aa, Homo sapiens
EVQLVESGGGLVQPGRSLRLSCAASGFTFDDYAMHWVRQAPGKGLEWVSGISWNSGSIGYADSVKGRFTISRDNAKKSLYLQMNSLRAEDTALYYCAKDSRGYGDYRLGGAYWGQGTLVTVSS

SEQ ID NO: 17 - protein, 123 aa, Homo sapiens
EVQLVESGGGLVQPGRSLRLSCEASGFTFDDYAMHWVRQAPGKGLEWVSGISWNSGSIGYADSVKGRFTISRDNAKNSLYLQMNSLRAEDTALYYCAKDSRGYGDYRLGGAYWGQGTLVTVSS

SEQ ID NO: 18 - protein, 123 aa, Homo sapiens
EVQLVESGGGLVQPGRSLRLSCAASGFTFDDYAMHWVRQAPGKGLEWVSGISWNSGSIGYADSVKGRFTISRDNAKNSLYLQMNSLRPEDTALYYCAKDSRGYGDYRLGGAYWGQGTLVTVSS

SEQ ID NO: 19 - protein, 107 aa, Homo sapiens
EIVMTQSPATLSVSPGERATLSCRASQSVSSNLAWYQQKPGQAPRLLIYGASTRATGIPARFSGSGSGTEFTLTISSLQSEDFAVYYCQQYNNWPWTFGQGTKVEIK

SEQ ID NO: 20 - protein, 243 aa, Homo sapiens
EVQLLESGGGLVQPGGSLRLSCAASGFTVSSYGMSWVRQAPGKGPEWVSGIRGSDGSTYYADSVKGRFTISRDNSKNTLYLQMNSLRAEDTAVYYCAKQGENDGPFDHRGQGTLVTVSSGGGGSEVQLLESGGGLVQPGGSLRLSCAASGFTVSSYGMSWVRQAPGKGPEWVSGIRGSDGSTYYADSVKGRFTISRDNSKNTLYLQMNSLRAEDTAVYYCAKQGENDGPFDHRGQGTLVTVSS

SEQ ID NO: 21 - protein, 119 aa, Homo sapiens
EVQLLESGGGLVQPGGSLRLSCAASGFTVSSYGMSWVRQAPGKGPEWVSGIRGSDGSTYYADSVKGRFTISRDNSKNTLYLQMNSLRAEDTAVYYCAKQGENDGPFDHRGQGTLVTVSS

SEQ ID NO: 22 - protein, 128 aa, H. sapiens
QLQLQESGPGLVKPSQTLSLTCTVSGGSISSGGHYWSWIRQHPGKGLEWIGYIHYSGSTYYNPSLKSRVIISVDTSKNQFSLKLRSVTAADTAVYYCARWRHDIFAAYPYYYYGMDVWGQGTLVTVSS